European Patent Specification EP 3 325 010 B1, published June 21, 2023. Title: ANTIBODIES TO COAGULATION FACTOR XIA AND USES THEREOF. Applicant: The Regents of the University of California Pfizer Inc. The sequence listing filed with the application follows.

SEQUENCE LISTING (103 sequences)

SEQ ID NO: 1 - protein, 117 aa, Artificial Sequence
  Synthetic construct
EVQLVQSGAEVKKPGASVKVSCKASGYTFTGYYMHWVRQAPGQGLEWMGWIDPDEGDTNYAQKFQGRVTMTRDTSISTAYMELSRLRSDDTAVYYCARLASGFRDYWGQGTLVTVSS

SEQ ID NO: 2 - protein, 5 aa, Artificial Sequence
  Synthetic Construct
GYYMH

SEQ ID NO: 3 - protein, 17 aa, Artificial Sequence
  Synthetic Construct
WIDPDEGDTNYAQKFQG

SEQ ID NO: 4 - protein, 8 aa, Artificial Sequence
  Synthetic Construct
LASGFRDY

SEQ ID NO: 5 - protein, 10 aa, Artificial Sequence
  Synthetic Construct
GYTFTGYYMH

SEQ ID NO: 6 - protein, 8 aa, Artificial Sequence
  Synthetic Construct
WIDPDEGD

SEQ ID NO: 7 - protein, 108 aa, Artificial Sequence
  Synthetic Construct
DIVMTKSPSSLSASVGDRVTITCRASQGIRNDLGWYQQKPGKAPKRLIYAASSLQSGVPSRFSGSGSGTEFTLTISSLQPEDFATYYCLQHDIYASTFGPGTKVDIKR

SEQ ID NO: 8 - protein, 11 aa, Artificial Sequence
  Synthetic Construct
RASQGIRNDLG

SEQ ID NO: 9 - protein, 8 aa, Artificial Sequence
  Synthetic Construct
YAASSLQS

SEQ ID NO: 10 - protein, 9 aa, Artificial Sequence
  Synthetic Construct
LQHDIYAST

SEQ ID NO: 11 - protein, 9 aa, Artificial Sequence
  Synthetic Construct
ASQGIRNDL

SEQ ID NO: 12 - protein, 5 aa, Artificial Sequence
  Synthetic Construct
YAASS

SEQ ID NO: 13 - protein, 8 aa, Artificial Sequence
  Synthetic Construct
QHDIYAST

SEQ ID NO: 14 - protein, 117 aa, Artificial Sequence
  Synthetic Construct
EVQLVQSGAEVKKPGASVKVSCKASGYTFTGYYMHWVRQAPGQGLEWMGWINPNSGGTNYAQKFQGRVTMTRDTSISTAYMELSRLRSDDTAVYYCARLASGFRDYWGQGTLVTVSS

SEQ ID NO: 15 - protein, 17 aa, Artificial Sequence
  Synthetic Construct
WINPNSGGTNYAQKFQG

SEQ ID NO: 16 - protein, 8 aa, Artificial Sequence
  Synthetic Construct
WINPNSGG

SEQ ID NO: 17 - protein, 108 aa, Artificial Sequence
  Synthetic Construct
DIVMTQSPSSLSASVGDRVTITCRASQGIRNDLGWYQQKPGKAPKRLIYAASSLQSGVPSRFSGSGSGTEFTLTISSLQPEDFATYYCLQHDIYASTFGPGTKVDIKR

SEQ ID NO: 18 - protein, 117 aa, Artificial Sequence
  Synthetic Construct
EVQLVQSGAEVKKPGASVKVSCKASGYTFTGYYMHWVRQAPGQGLEWMGRINPNSGDTNYAQKFQGRVTMTRDTSISTAYMELSRLRSDDTAVYYCARLASGFRDYWGQGTLVTVSS

SEQ ID NO: 19 - protein, 17 aa, Artificial Sequence
  Synthetic Construct
RINPNSGDTNYAQKFQG

SEQ ID NO: 20 - protein, 8 aa, Artificial Sequence
  Synthetic Construct
RINPNSGD

SEQ ID NO: 21 - protein, 108 aa, Artificial Sequence; identical to SEQ ID NO: 17
  Synthetic anti-FXIa antibody QCA11_VL AA

SEQ ID NO: 22 - protein, 117 aa, Artificial Sequence
  Synthetic Construct
EVQLVQSGAEVKKPGASVKVSCKASGYTFTGYYMHWVRQAPGQGLEWMGWINPNSGGTNYAQKFQGRVTMTRDTSISTAYMELSRLSSDDTAVYYCARLASGFRDYWGQGTLVTVSS

SEQ ID NO: 23 - protein, 108 aa, Artificial Sequence; identical to SEQ ID NO: 17
  Synthetic Construct

SEQ ID NO: 24 - protein, 117 aa, Artificial Sequence; identical to SEQ ID NO: 14
  Synthetic Construct

SEQ ID NO: 25 - protein, 108 aa, Artificial Sequence
  Synthetic Construct
DIVMTQSPSSLSASVGDRVTITCRASQGIRNDLGWYQQKPGKAPKRLIYAASSLQSGVPSRFSGSVSGTEFTLTISSLQPEDLATYYCLQHDIYASTFGPGTKVDIKR

SEQ ID NO: 26 - protein, 117 aa, Artificial Sequence; identical to SEQ ID NO: 14
  Synthetic Construct

SEQ ID NO: 27 - protein, 108 aa, Artificial Sequence; identical to SEQ ID NO: 17
  Synthetic Construct

SEQ ID NO: 28 - protein, 117 aa, Artificial Sequence
  Synthetic Construct
EVQLVQSGAEVKKPGASVKVSCKASGYTFTGYYMHWVRQAPGQGLEWMGRINPNSGGTNYAQKFQGRVTMTRDTSISTAYMELSRLRSDDTAVYYCARLASGFRDYWGQGTLVTVSS

SEQ ID NO: 29 - protein, 17 aa, Artificial Sequence
  Synthetic Construct
RINPNSGGTNYAQKFQG

SEQ ID NO: 30 - protein, 8 aa, Artificial Sequence
  Synthetic Construct
RINPNSGG

SEQ ID NO: 31 - protein, 108 aa, Artificial Sequence
  Synthetic Construct
DIVMTQSPSSLSASVGDRVTITCRASLGIRNDLGWYQQKPGKAPKRLIYAASSLQSGVPSRFSGSGSGTEFSLTISSLQPEDFATYYCLQHDIYASTFGPGTKVDIKR

SEQ ID NO: 32 - protein, 11 aa, Artificial Sequence
  Synthetic Construct
RASLGIRNDLG

SEQ ID NO: 33 - protein, 9 aa, Artificial Sequence
  Synthetic Construct
ASLGIRNDL

SEQ ID NO: 34 - protein, 117 aa, Artificial Sequence
  Synthetic Construct
EVQLVQSGAEVKKPGASVKVSCKASGYTFTGYYMHWVRQAPGQGLEWMGWIDPNSGDTNYAQKFQGRVTMTRDTSISTAYMELSRLRSDDTAVYYCARLASGFRDYWGQGTLVTVSS

SEQ ID NO: 35 - protein, 17 aa, Artificial Sequence
  Synthetic Construct
WIDPNSGDTNYAQKFQG

SEQ ID NO: 36 - protein, 8 aa, Artificial Sequence
  Synthetic Construct
WIDPNSGD

SEQ ID NO: 37 - protein, 108 aa, Artificial Sequence; identical to SEQ ID NO: 17
  Synthetic Construct

SEQ ID NO: 38 - protein, 117 aa, Artificial Sequence; identical to SEQ ID NO: 14
  Synthetic Construct

SEQ ID NO: 39 - protein, 108 aa, Artificial Sequence; identical to SEQ ID NO: 7
  Synthetic Construct

SEQ ID NO: 40 - protein, 117 aa, Artificial Sequence
  Synthetic Construct
EVQLVQSGAEVKKPGASVKVSCKASGYTFTGYYMHWVRQAPGQGLEWMGWINPNSGGTNYAPKFQGRVTMTRDTSISTAYMELSRLRSDDTAVYYCARLASGFRDYWGQGTLVTVSS

SEQ ID NO: 41 - protein, 17 aa, Artificial Sequence
  Synthetic Construct
WINPNSGGTNYAPKFQG

SEQ ID NO: 42 - protein, 108 aa, Artificial Sequence
  Synthetic Construct
DIVMTQSPSSLSASVGDRVTITCRASQGIRNDLGWYQQKPGKAPKRLIYAASSLQSGVPSRFSGSASGTEFTLTISSLQPEDFATYYCLQHDIYASTFGPGTKVDIKR

SEQ ID NO: 43 - protein, 117 aa, Artificial Sequence
  Synthetic Construct
EVQLVQSGAEVKKPGASVKVSCKASGYTFTGYYMHWVRQAPGQGLEWMGWIDPDSGGTNYAQKFQGRVTMTRDTSISTAYMELSRLRSDDTAVYYCARLASGFRDYWGHGTLVTVSS

SEQ ID NO: 44 - protein, 17 aa, Artificial Sequence
  Synthetic Construct
WIDPDSGGTNYAQKFQG

SEQ ID NO: 45 - protein, 8 aa, Artificial Sequence
  Synthetic Construct
WIDPDSGG

SEQ ID NO: 46 - protein, 108 aa, Artificial Sequence; identical to SEQ ID NO: 17
  Synthetic Construct

SEQ ID NO: 47 - protein, 117 aa, Artificial Sequence
  Synthetic Construct
EVQLVQSGAEVKKPGASVKVSCKASGYTFTGYYMHWVRQAPGQGLEWMGWIDPDSGDTNYAQKFQGRVTMTRDTSISTAYMELSRLRSDDTAVYYCARLASGFRDYWGQGTLVTVSS

SEQ ID NO: 48 - protein, 17 aa, Artificial Sequence
  Synthetic Construct
WIDPDSGDTNYAQKFQG

SEQ ID NO: 49 - protein, 7 aa, Artificial Sequence
  Synthetic Construct
WIDPDSG

SEQ ID NO: 50 - protein, 108 aa, Artificial Sequence; identical to SEQ ID NO: 17
  Synthetic Construct

SEQ ID NO: 51 - protein, 117 aa, Artificial Sequence
  Synthetic Construct
EVQLVQSGAEVKKPGASVKVSCKASGYTFTGYYMHWVRQAPGQGLEWMGRIDPDSGDTNYAQKFQGRVTMTRDTSISTAYMELSRLRSDDTAVYYCARLASGFRDYWGQGTLVTVSS

SEQ ID NO: 52 - protein, 17 aa, Artificial Sequence
  Synthetic Construct
RIDPDSGDTNYAQKFQG

SEQ ID NO: 53 - protein, 8 aa, Artificial Sequence
  Synthetic Construct
RIDPDSGD

SEQ ID NO: 54 - protein, 108 aa, Artificial Sequence; identical to SEQ ID NO: 17
  Synthetic Construct

SEQ ID NO: 55 - protein, 117 aa, Artificial Sequence
  Synthetic Construct
EVQLVQSGAEVKKPGASVKVSCKASGYTFTGYYMHWVRQAPGQGLEWMGWINPDSGDTNYAQKFQGRVTMTRDTSISTAYMELSRLRSDDTAVYYCARLASGFRDYWGQGTLVTVSS

SEQ ID NO: 56 - protein, 17 aa, Artificial Sequence
  Synthetic Construct
WINPDSGDTNYAQKFQG

SEQ ID NO: 57 - protein, 8 aa, Artificial Sequence
  Synthetic Construct
WINPDSGD

SEQ ID NO: 58 - protein, 108 aa, Artificial Sequence; identical to SEQ ID NO: 7
  Synthetic Construct

SEQ ID NO: 59 - protein, 117 aa, Artificial Sequence; identical to SEQ ID NO: 34
  Synthetic Construct

SEQ ID NO: 60 - protein, 17 aa, Artificial Sequence
  Synthetic Construct
WIDPNSGDTNYAQKFQG

SEQ ID NO: 61 - protein, 8 aa, Artificial Sequence
  Synthetic Construct
WIDPNSGD

SEQ ID NO: 62 - protein, 108 aa, Artificial Sequence; identical to SEQ ID NO: 7
  Synthetic Construct

SEQ ID NO: 63 - protein, 117 aa, Artificial Sequence; identical to SEQ ID NO: 51
  Synthetic Construct

SEQ ID NO: 64 - protein, 108 aa, Artificial Sequence; identical to SEQ ID NO: 7
  Synthetic Construct

SEQ ID NO: 65 - protein, 117 aa, Artificial Sequence; identical to SEQ ID NO: 47
  Synthetic Construct

SEQ ID NO: 66 - protein, 17 aa, Artificial Sequence
  Synthetic Construct
WIDPDSGDTNYAQKFQG

SEQ ID NO: 67 - protein, 8 aa, Artificial Sequence
  Synthetic Construct
WIDPDSGD

SEQ ID NO: 68 - protein, 108 aa, Artificial Sequence; identical to SEQ ID NO: 7
  Synthetic Construct

SEQ ID NO: 69 - protein, 122 aa, Artificial Sequence
  Synthetic Construct
QVQLVQSGAEVKKPGASVKVSCKASGYTFTSYYMHWVRQAPGQGLEWMGIINPSGGSTSYAQKFQGRVTMTRDTSTSTVYMELSSLRSEDTAVYYCARDTIPGIAVAGTDYWGQGTLVTVSS

SEQ ID NO: 70 - protein, 5 aa, Artificial Sequence
  Synthetic Construct
SYYMH

SEQ ID NO: 71 - protein, 17 aa, Artificial Sequence
  Synthetic Construct
IINPSGGSTSYAQKFQG

SEQ ID NO: 72 - protein, 13 aa, Artificial Sequence
  Synthetic Construct
DTIPGIAVAGTDY

SEQ ID NO: 73 - protein, 10 aa, Artificial Sequence
  Synthetic Construct
GYTFTSYYMH

SEQ ID NO: 74 - protein, 8 aa, Artificial Sequence
  Synthetic Construct
IINPSGGS

SEQ ID NO: 75 - protein, 110 aa, Artificial Sequence
  Synthetic Construct
QSVLTQPPSVSAAPGQKVTISCSGSTSNIGNNYVSWYQQVPGTPPKLLIYDNDKRPSGIPDRFSGSKSGTSATLDITGLQTGDEADYYCGTWHSGLYVVVFGGGTKLTVL

SEQ ID NO: 76 - protein, 13 aa, Artificial Sequence
  Synthetic Construct
SGSTSNIGNNYVS

SEQ ID NO: 77 - protein, 8 aa, Artificial Sequence
  Synthetic Construct
YDNDKRPS

SEQ ID NO: 78 - protein, 11 aa, Artificial Sequence
  Synthetic Construct
GTWHSGLYVVV

SEQ ID NO: 79 - protein, 11 aa, Artificial Sequence
  Synthetic Construct
GSTSNIGNNYV

SEQ ID NO: 80 - protein, 5 aa, Artificial Sequence
  Synthetic Construct
YDNDK

SEQ ID NO: 81 - protein, 10 aa, Artificial Sequence
  Synthetic Construct
TWHSGLYVVV

SEQ ID NO: 82 - protein, 330 aa, Artificial Sequence
  Synthetic Construct
ASTKGPSVFPLAPSSKSTSGGTAALGCLVKDYFPEPVTVSWNSGALTSGVHTFPAVLQSSGLYSLSSVVTVPSSSLGTQTYICNVNHKPSNTKVDKKVEPKSCDKTHTCPPCPAPEAAGAPSVFLFPPKPKDTLMISRTPEVTCVVVDVSHEDPEVKFNWYVDGVEVHNAKTKPREEQYNSTYRVVSVLTVLHQDWLNGKEYKCKVSNKALPAPIEKTISKAKGQPREPQVYTLPPSREEMTKNQVSLTCLVKGFYPSDIAVEWESNGQPENNYKTTPPVLDSDGSFFLYSKLTVDKSRWQQGNVFSCSVMHEALHNHYTQKSLSLSPGK

SEQ ID NO: 83 - protein, 106 aa, Artificial Sequence
  Synthetic Construct
TVAAPSVFIFPPSDEQLKSGTASVVCLLNNFYPREAKVQWKVDNALQSGNSQESVTEQDSKDSTYSLSSTLTLSKADYEKHKVYACEVTHQGLSSPVTKSFNRGEC

SEQ ID NO: 84 - DNA, 351 bp, Artificial Sequence
  Synthetic Construct
gaggtccagctggtgcagtctggggctgaggtgaagaagcctggggcctcagtgaaggtctcctgcaaggcttctggatacaccttcaccggctactatatgcactgggtgcgacaggcccctggacaagggcttgagtggatgggatggatcgaccctgacgaaggtgacacaaactatgcacagaagtttcagggcagggtcaccatgaccagggacacgtccatcagcacagcctacatggagctgagcaggctgagatctgacgacacggccgtgtattactgtgcgagattagctagtggctttcgtgactactggggccagggaaccctggtcaccgtctcgagc

SEQ ID NO: 85 - DNA, 324 bp, Artificial Sequence
  Synthetic Construct
gacatcgtgatgaccaagtctccatcctccctgtctgcttctgtaggagacagagtcaccatcacttgccgggcaagtcagggcattagaaatgatttaggctggtatcagcagaaaccagggaaagcccctaagcgcctcatctatgctgcatccagtttgcaaagtggggtcccatcaaggttcagcggcagtggatctgggacagaattcactctcacaatcagcagcctgcagcctgaagattttgcaacttattactgtctacagcatgatatttacgctagcactttcggccctgggaccaaagtggatatcaaacgt

SEQ ID NO: 86 - DNA, 351 bp, Artificial Sequence
  Synthetic Construct
gaggtccagctggtgcagtctggggctgaggtgaagaagcctggggcctcagtgaaggtctcctgcaaggcttctggatacaccttcaccggctactatatgcactgggtgcgacaggcccctggacaagggcttgagtggatgggatggatcaaccctaacagtggtggcacaaactatgcacagaagtttcagggcagggtcaccatgaccagggacacgtccatcagcacagcctacatggagctgagcaggctgagatctgacgacacggccgtgtattactgtgcgagattagctagtggctttcgtgactactggggccagggaaccctggtcaccgtctcgagc

SEQ ID NO: 87 - DNA, 324 bp, Artificial Sequence
  Synthetic Construct
gacatcgtgatgacccagtctccatcctccctgtctgcatctgtaggagacagagtcaccatcacttgccgggcaagtcagggcattagaaatgatttaggctggtatcagcagaaaccagggaaagcccctaagcgcctcatctatgctgcatccagtttgcaaagtggggtcccatcaaggttcagcggcagtggatctgggacagaattcactctcacaatcagcagcctgcagcctgaagattttgcaacttattactgtctacagcatgatatttacgctagcactttcggccctgggaccaaagtggatatcaaacgt

SEQ ID NO: 88 - DNA, 351 bp, Artificial Sequence
  Synthetic Construct
gaggtccagctggtgcagtctggggctgaggtgaagaagcctggggcctcagtgaaggtctcctgcaaggcttctggatacaccttcaccggctactatatgcactgggtgcgacaggcccctggacaagggcttgagtggatgggatggatcgaccctgacagtggtgacacaaactatgcacagaagtttcagggcagggtcaccatgaccagggacacgtccatcagcacagcctacatggagctgagcaggctgagatctgacgacacggccgtgtattactgtgcgagattagctagtggctttcgtgactactggggccagggaaccctggtcaccgtctcgagc

SEQ ID NO: 89 - DNA, 324 bp, Artificial Sequence; identical to SEQ ID NO: 85
  Synthetic Construct

SEQ ID NO: 90 - DNA, 366 bp, Artificial Sequence
  Synthetic Construct
caggtccagctggtacagtctggggctgaggtgaagaagcctggggcctcagtgaaggtttcctgcaaggcatctggatacaccttcaccagctactatatgcactgggtgcgacaggcccctggacaagggcttgagtggatgggaataatcaaccctagtggtggtagcacaagctacgcacagaagttccagggcagagtcaccatgaccagggacacgtccacgagcacagtctacatggagctgagcagcctgagatctgaggacacggccgtgtattactgtgcgagagacactattccgggtatagcagtggctggtacggactactggggccagggaaccctggtcaccgtctcgagc

SEQ ID NO: 91 - DNA, 330 bp, Artificial Sequence
  Synthetic Construct
cagtctgtcttgacgcagccgccctcagtgtctgcggccccaggacagaaggtcaccatctcctgctctggaagcacctccaacattggcaataattatgtatcctggtaccagcaggtcccaggaacaccccccaaactcctcatttatgacaatgataagcgaccctcagggattcctgaccgattctctggctccaagtctggcacgtcagccaccctggacatcaccggactccagactggggacgaggccgattattactgcggaacatggcatagtggcctgtatgtcgtggtgttcggcggagggaccaagctgaccgtccta

SEQ ID NO: 92 - DNA, 990 bp, Artificial Sequence
  Synthetic Construct
gcctccaccaagggcccatcggtcttccccctggcaccctcctccaagagcacctctgggggcacagcggccctgggctgcctggtcaaggactacttccccgaaccggtgacggtgtcgtggaactcaggcgccctgaccagcggcgtgcacaccttcccggctgtcctacagtcctcaggactctactccctcagcagcgtggtgaccgtgccctccagcagcttgggcacccagacctacatctgcaacgtgaatcacaagcccagcaacaccaaggtggacaagaaagttgagcccaaatcttgtgacaaaactcacacatgcccaccgtgcccagcacctgaagccgctggggcaccgtcagtcttcctcttccccccaaaacccaaggacaccctcatgatctcccggacccctgaggtcacatgcgtggtggtggacgtgagccacgaagaccctgaggtcaagttcaactggtacgtggacggcgtggaggtgcataatgccaagacaaagccgcgggaggagcagtacaacagcacgtaccgtgtggtcagcgtcctcaccgtcctgcaccaggactggctgaatggcaaggagtacaagtgcaaggtctccaacaaagccctcccagcccccatcgagaaaaccatctccaaagccaaagggcagccccgagaaccacaggtgtacaccctgcccccatcccgggaggagatgaccaagaaccaggtcagcctgacctgcctggtcaaaggcttctatcccagcgacatcgccgtggagtgggagagcaatgggcagccggagaacaactacaagaccacgcctcccgtgctggactccgacggctccttcttcctctatagcaagctcaccgtggacaagagcaggtggcagcaggggaacgtcttctcatgctccgtgatgcatgaggctctgcacaaccactacacgcagaagagcctctccctgtctccgggtaaa

SEQ ID NO: 93 - DNA, 318 bp, Artificial Sequence
  Synthetic Construct
actgtggctgcaccatctgtcttcatcttcccgccatctgatgagcagttgaaatctggaactgcctctgttgtgtgcctgctgaataacttctatcccagagaggccaaagtacagtggaaggtggataacgccctccaatcgggtaactcccaggagagtgtcacagagcaggacagcaaggacagcacctacagcctcagcagcaccctgacgctgagcaaagcagactacgagaaacacaaagtctacgcctgcgaagtcacccatcagggcctgagctcgcccgtcacaaagagcttcaacaggggagagtgt

SEQ ID NO: 94 - protein, 17 aa, Artificial Sequence
  Synthetic Construct
  VARIANT (1)..(1): Xaa = Trp or Arg
  VARIANT (3)..(3): Xaa = Asn or Asp
  VARIANT (5)..(5): Xaa = Asn or Asp
  VARIANT (6)..(6): Xaa = Ser or Glu
  VARIANT (8)..(8): Xaa = Gly or Asp
  VARIANT (13)..(13): Xaa = Gln or Pro
XIXPXXGXTNYAXKFQG

SEQ ID NO: 95 - protein, 8 aa, Artificial Sequence
  Synthetic Construct
  VARIANT (1)..(1): Xaa = Trp or Arg
  VARIANT (3)..(3): Xaa = Asn or Asp
  VARIANT (5)..(5): Xaa = Asn or Asp
  VARIANT (6)..(6): Xaa = Ser or Glu
  VARIANT (8)..(8): Xaa = Gly or Asp
XIXPXXGX

SEQ ID NO: 96 - protein, 117 aa, Artificial Sequence
  Synthetic Construct
  VARIANT (50)..(50): Xaa = Trp or Arg
  VARIANT (52)..(52): Xaa = Asn or Asp
  VARIANT (54)..(54): Xaa = Asn or Asp
  VARIANT (55)..(55): Xaa =  Ser or Glu
  VARIANT (57)..(57): Xaa =  Gly or Asp
  VARIANT (62)..(62): Xaa =  Gln or Pro
  VARIANT (87)..(87): Xaa =  Arg or Ser
  VARIANT (109)..(109): Xaa =  Gln or His
EVQLVQSGAEVKKPGASVKVSCKASGYTFTGYYMHWVRQAPGQGLEWMGXIXPXXGXTNYAXKFQGRVTMTRDTSISTAYMELSRLXSDDTAVYYCARLASGFRDYWGXGTLVTVSS

SEQ ID NO: 97 - protein, 108 aa, Artificial Sequence
  Synthetic Construct
  VARIANT (6)..(6): Xaa = Gln  or Lys
  VARIANT (27)..(27): Xaa = Gln  or Leu
  VARIANT (66)..(66): Xaa = Gly, Val or Ala
  VARIANT (72)..(72): Xaa = Thr or Ser
  VARIANT (83)..(83): Xaa = Phe or Leu
DIVMTXSPSSLSASVGDRVTITCRASXGIRNDLGWYQQKPGKAPKRLIYAASSLQSGVPSRFSGSXSGTEFXLTISSLQPEDXATYYCLQHDIYASTFGPGTKVDIKR

SEQ ID NO: 98 - protein, 625 aa, Homo sapiens
MIFLYQVVHFILFTSVSGECVTQLLKDTCFEGGDITTVFTPSAKYCQVVCTYHPRCLLFTFTAESPSEDPTRWFTCVLKDSVTETLPRVNRTAAISGYSFKQCSHQISACNKDIYVDLDMKGINYNSSVAKSAQECQERCTDDVHCHFFTYATRQFPSLEHRNICLLKHTQTGTPTRITKLDKVVSGFSLKSCALSNLACIRDIFPNTVFADSNIDSVMAPDAFVCGRICTHHPGCLFFTFFSQEWPKESQRNLCLLKTSESGLPSTRIKKSKALSGFSLQSCRHSIPVFCHSSFYHDTDFLGEELDIVAAKSHEACQKLCTNAVRCQFFTYTPAQASCNEGKGKCYLKLSSNGSPTKILHGRGGISGYTLRLCKMDNECTTKIKPRIVGGTASVRGEWPWQVTLHTTSPTQRHLCGGSIIGNQWILTAAHCFYGVESPKILRVYSGILNQSEIKEDTSFFGVQEIIIHDQYKMAESGYDIALLKLETTVNYTDSQRPICLPSKGDRNVIYTDCWVTGWGYRKLRDKIQNTLQKAKIPLVTNEECQKRYRGHKITHKMICAGYREGGKDACKGDSGGPLSCKHNEVWHLVGITSWGEGCAQRERPGVYTNVVEYVDWILEKTQAV

SEQ ID NO: 99 - protein, 262 aa, Artificial Sequence
  Synthetic Construct
MGWSCIILFLVATATGVHSIVGGTASVRGEWPWQVTLHTTSPTQRHLCGGSIIGNQWILTAAHCFYGVESPKILRVYSGILQQSEIKEDTSFFGVQEIIIHDQYKMAESGYDIALLKLETTVQYTDSQRPISLPSKGDRNVIYTDCWVTGWGYRKLRDKIQNTLQKAKIPLVTNEECQKRYRGHKITHKMICAGYREGGKDACKGDAGGPLSCKHNEVWHLVGITSWGEGCAQRERPGVYTNVVEYVDWILEKTQAHHHHHH

SEQ ID NO: 100 - protein, 243 aa, Artificial Sequence
  Synthetic Construct
IVGGTASVRGEWPWQVTLHTTSPTQRHLCGGSIIGNQWILTAAHCFYGVESPKILRVYSGILQQSEIKEDTSFFGVQEIIIHDQYKMAESGYDIALLKLETTVQYTDSQRPISLPSKGDRNVIYTDCWVTGWGYRKLRDKIQNTLQKAKIPLVTNEECQKRYRGHKITHKMICAGYREGGKDACKGDAGGPLSCKHNEVWHLVGITSWGEGCAQRERPGVYTNVVEYVDWILEKTQAHHHHHH

SEQ ID NO: 101 - protein, 229 aa, Artificial Sequence
  Synthetic Construct
EVQLVQSGAEVKKPGASVKVSCKASGYTFTGYYMHWVRQAPGQGLEWMGWIDPDEGDTNYAQKFQGRVTMTRDTSISTAYMELSRLRSDDTAVYYCARLASGFRDYWGQGTLVTVSSASTKGPSVFPLAPSSKSTSGGTAALGCLVKDYFPEPVTVSWNSGALTSGVHTFPAVLQSSGLYSLSSVVTVPSSSLGTQTYICNVNHKPSNTKVDKKVEPKSCGGSHHHHHH

SEQ ID NO: 102 - protein, 213 aa, Artificial Sequence
  Synthetic Construct
DIVMTKSPSSLSASVGDRVTITCRASQGIRNDLGWYQQKPGKAPKRLIYAASSLQSGVPSRFSGSGSGTEFTLTISSLQPEDFATYYCLQHDIYASTFGPGTKVDIKTVAAPSVFIFPPSDEQLKSGTASVVCLLNNFYPREAKVQWKVDNALQSGNSQESVTEQDSKDSTYSLSSTLTLSKADYEKHKVYACEVTHQGLSSPVTKSFNRGEC

SEQ ID NO: 103 - protein, 330 aa, Artificial Sequence
  Synthetic Construct
ASTKGPSVFPLAPSSKSTSGGTAALGCLVKDYFPEPVTVSWNSGALTSGVHTFPAVLQSSGLYSLSSVVTVPSSSLGTQTYICNVNHKPSNTKVDKKVEPKSCDKTHTCPPCPAPELLGGPSVFLFPPKPKDTLMISRTPEVTCVVVDVSHEDPEVKFNWYVDGVEVHNAKTKPREEQYNSTYRVVSVLTVLHQDWLNGKEYKCKVSNKALPAPIEKTISKAKGQPREPQVYTLPPSREEMTKNQVSLTCLVKGFYPSDIAVEWESNGQPENNYKTTPPVLDSDGSFFLYSKLTVDKSRWQQGNVFSCSVMHEALHNHYTQKSLSLSPGK